European Patent Specification EP 3 950 718 B1, published January 7, 2026. Title: Genetically Engineered Dual-targeting Chimeric Antigen Receptor and Use Thereof. Applicant: West China Hospotal,Sichuan University. The sequence listing filed with the application follows.

SEQUENCE LISTING (26 sequences)

SEQ ID NO: 1 - protein, 373 aa, Artificial Sequence
DIQMTQSPSSLSASVGDRVTITCRASQDVSTAVAWYQQKPGKAPKLLIYSASFLYSGVPSRFSGSGSGTDFTLTISSLQPEDFATYYCQQYLYHPATFGQGTKVEIKGGGGSGGGGSGGGGSEVQLVESGGGLVQPGGSLRLSCAASGFTFSDSWIHWVRQAPGKGLEWVAWISPYGGSTYYADSVKGRFTISADTSKNTAYLQMNSLRAEDTAVYYCARRHWPGGFDYWGQGTLVTVSAAAAFVPVFLPAKPTTTPAPRPPTPAPTIASQPLSLRPEACRPAAGGAVHTRGLDFACDIYIWAPLAGTCGVLLLSLVITLYCNHRNRFSVVKRGRKKLLYIFKQPFMRPVQTTQEEDGCSCRFPEEEEGGCEL

SEQ ID NO: 2 - DNA, 1122 bp, Artificial Sequence
gacatccaaatgacccagagccctagctccctgtccgctagcgtgggcgacagggtgaccatcacctgcagagccagccaggacgtgagcaccgccgtggcctggtaccagcagaagcccggcaaggcccccaagctgctgatctacagcgcctccttcctgtactccggcgtgccctccagatttagcggcagcggcagcggcacagacttcaccctcaccatcagctccctgcagcctgaggacttcgccacatactactgccagcagtacctctaccaccctgccaccttcggccaaggcaccaaggtggagatcaagggcggcggaggttctggcggaggcggctccggaggaggaggcagcgaagtgcagctggtggagagcggaggaggactggtgcagcctggcggaagcctgaggctgagctgtgctgccagcggcttcaccttctccgactcctggattcattgggtcaggcaggcccccggaaaaggactggagtgggtcgcctggatctccccttacggcggcagcacctactacgccgacagcgtgaagggcaggttcaccatcagcgccgataccagcaagaacaccgcctacctgcagatgaactccctgagggctgaggacaccgccgtgtactactgcgccaggaggcactggcctggcggattcgactactggggccagggcaccctggtgaccgtgtccgccgccgccgccttcgtgcctgtgtttctgcccgccaagcccaccaccacacctgctcccagacctcccacacctgcccctaccatcgctagccagcccctgagcctgagacccgaggcttgtaggcctgctgctggcggagccgtgcacacaagaggcctggacttcgcctgcgacatctacatctgggcccccctggccggaacatgtggagtgctgctgctgagcctggtgatcaccctgtactgcaaccacaggaacaggttcagcgtggtgaagaggggcaggaagaagctgctgtacatcttcaagcagcccttcatgaggcccgtgcagaccacccaggaggaggatggctgcagctgcaggttccctgaagaggaggagggcggctgcgagctgtga

SEQ ID NO: 3 - protein, 482 aa, Artificial Sequence
MALPVTALLLPLALLLHAARPEIVLTQSPGTLSLSPGERATLSCRASQSVSSSYLAWYQQKPGQAPRLLIYGASSRATGIPDRFSGSGSGTDFTLTISRLEPEDFAVYYCQQYGSSPLTFGGGTKVEIKGGGGSGGGGSGGGGSQAQVVESGGGVVQSGRSLRLSCAASGFAFSSYGMHWVRQAPGKGLEWVAVIWYDGSNKYYADSVRGRFTISRDNSENTLYLQMNSLRAEDTAVYYCARDHYGSGVHHYFYYGLDVWGQGTTVTVSSKIEVMYPPPYLDNEKSNGTIIHVKGKHLCPSPLFPGPSKPFWVLVVVGGVLACYSLLVTVAFIIFWVRSKRSRLLHSDYMNMTPRRPGPTRKHYQPYAPPRDFAAYRSAPAYQQGQNQLYNELNLGRREEYDVLDKRRGRDPEMGGKPQRRKNPQEGLYNELQKDKMAEAYSEIGMKGERRRGKGHDGLYQGLSTATKDTYDALHMQALPPR

SEQ ID NO: 4 - DNA, 1446 bp, Artificial Sequence
atggccttaccagtgaccgccttgctcctgccgctggccttgctgctccacgccgccaggccggagatcgtgctgacacagagccctggcaccctgagcctgtcccccggcgaaagagccaccctgtcctgcagagccagccagagcgtgagcagctcctatctggcctggtaccagcagaagcctggccaggcccccagactcctgatctacggcgccagcagcagagccaccggcatccccgatagattcagcggctccggcagcggaaccgactttaccctgaccatctccagactggagcccgaggactttgccgtgtactactgccagcagtacggcagcagccccctgacattcggcggcggcacaaaggtggagatcaaaggcggcggaggttctggaggaggaggaagcggaggaggaggcagccaggctcaggtggtcgaaagcggcggaggagtggtgcagagcggaaggtccctgaggctgagctgcgctgctagcggctttgccttctcctcctacggcatgcactgggtgagacaggcccctggcaagggcctggaatgggtggctgtgatctggtacgacggcagcaacaagtactacgccgacagcgtgaggggcaggttcaccatcagcagggacaacagcgaaaacaccctgtacctgcagatgaacagcctcagggccgaggataccgccgtgtattattgcgccagggatcactacggaagcggcgtgcaccattacttctattacggcctggacgtgtggggccagggcacaacagtgaccgtgtccagcaaaattgaagttatgtatcctcctccttacctagacaatgagaagagcaatggaaccattatccatgtgaaagggaaacacctttgtccaagtcccctatttcccggaccttctaagcccttttgggtgctggtggtggttggtggagtcctggcttgctatagcttgctagtaacagtggcctttattattttctgggtgaggagtaagaggagcaggctcctgcacagtgactacatgaacatgactccccgccgccccgggcccacccgcaagcattaccagccctatgccccaccacgcgacttcgcagcctatcgctccgcccccgcgtaccagcagggccagaaccagctctataacgagctcaatctaggacgaagagaggagtacgatgttttggacaagagacgtggccgggaccctgagatggggggaaagccgcagagaaggaagaaccctcaggaaggcctgtacaatgaactgcagaaagataagatggcggaggcctacagtgagattgggatgaaaggcgagcgccggaggggcaaggggcacgatggcctttaccagggtctcagtacagccaccaaggacacctacgacgcccttcacatgcaggccctgccccctcgc

SEQ ID NO: 5 - protein, 475 aa, Artificial Sequence
MALPVTALLLPLALLLHAARPMQVQLQQSGPELKKPGETVKISCKASGYPFTNYGMNWVKQAPGQGLKWMGWINTSTGESTFADDFKGRFDFSLETSANTAYLQINNLKSEDSATYFCARWEVYHGYVPYWGQGTTVTVSSGGGGSGGGGSGGGGSDIQLTQSHKFLSTSVGDRVSITCKASQDVYNAVAWYQQKPGQSPKLLIYSASSRYTGVPSRFTGSGSGPDFTFTISSVQAEDLAVYFCQQHFRTPFTFGSGTKLEIKKIEVMYPPPYLDNEKSNGTIIHVKGKHLCPSPLFPGPSKPFWVLVVVGGVLACYSLLVTVAFIIFWVRSKRSRLLHSDYMNMTPRRPGPTRKHYQPYAPPRDFAAYRSAPAYQQGQNQLYNELNLGRREEYDVLDKRRGRDPEMGGKPQRRKNPQEGLYNELQKDKMAEAYSEIGMKGERRRGKGHDGLYQGLSTATKDTYDALHMQALPPR

SEQ ID NO: 6 - DNA, 1428 bp, Artificial Sequence
atggccttaccagtgaccgccttgctcctgccgctggccttgctgctccacgccgccaggccgatgcaggtacaactgcagcagtcaggacctgaactgaagaagcctggagagacagtcaagatctcctgcaaggcctctgggtatcctttcacaaactatggaatgaactgggtgaagcaggctccaggacagggtttaaagtggatgggctggattaacacctccactggagagtcaacatttgctgatgacttcaagggacggtttgacttctctttggaaacctctgccaacactgcctatttgcagatcaacaacctcaaaagtgaagactcggctacatatttctgtgcaagatgggaggtttaccacggctacgttccttactggggccaagggaccacggtcaccgtttcctctggcggtggcggttctggtggcggtggctccggcggtggcggttctgacatccagctgacccagtctcacaaattcctgtccacttcagtaggagacagggtcagcatcacctgcaaggccagtcaggatgtgtataatgctgttgcctggtatcaacagaaaccaggacaatctcctaaacttctgatttactcggcatcctcccggtacactggagtcccttctcgcttcactggcagtggctctgggccggatttcactttcaccatcagcagtgtgcaggctgaagacctggcagtttatttctgtcagcaacattttcgtactccattcacgttcggctcggggacaaaattggagatcaaaaaaattgaagttatgtatcctcctccttacctagacaatgagaagagcaatggaaccattatccatgtgaaagggaaacacctttgtccaagtcccctatttcccggaccttctaagcccttttgggtgctggtggtggttggtggagtcctggcttgctatagcttgctagtaacagtggcctttattattttctgggtgaggagtaagaggagcaggctcctgcacagtgactacatgaacatgactccccgccgccccgggcccacccgcaagcattaccagccctatgccccaccacgcgacttcgcagcctatcgctccgcccccgcgtaccagcagggccagaaccagctctataacgagctcaatctaggacgaagagaggagtacgatgttttggacaagagacgtggccgggaccctgagatggggggaaagccgcagagaaggaagaaccctcaggaaggcctgtacaatgaactgcagaaagataagatggcggaggcctacagtgagattgggatgaaaggcgagcgccggaggggcaaggggcacgatggcctttaccagggtctcagtacagccaccaaggacacctacgacgcccttcacatgcaggccctgccccctcgctaa

SEQ ID NO: 7 - protein, 22 aa, Artificial Sequence
SGSGEGRGSLLTCGDVEENPGP

SEQ ID NO: 8 - DNA, 66 bp, Artificial Sequence
agcggcagcggcgagggaagaggaagcctgctgacctgcggcgatgtggaggagaatcccggcccc

SEQ ID NO: 9 - protein, 4 aa, Artificial Sequence
RRKR

SEQ ID NO: 10 - DNA, 12 bp, Artificial Sequence
aggaggaagaga

SEQ ID NO: 11 - protein, 21 aa, Artificial Sequence
MALPVTALLLPLALLLHAARP

SEQ ID NO: 12 - DNA, 63 bp, Artificial Sequence
atggccttaccagtgaccgccttgctcctgccgctggccttgctgctccacgccgccaggccg

SEQ ID NO: 13 - protein, 242 aa, Artificial Sequence
MQVQLQQSGPELKKPGETVKISCKASGYPFTNYGMNWVKQAPGQGLKWMGWINTSTGESTFADDFKGRFDFSLETSANTAYLQINNLKSEDSATYFCARWEVYHGYVPYWGQGTTVTVSSGGGGSGGGGSGGGGSDIQLTQSHKFLSTSVGDRVSITCKASQDVYNAVAWYQQKPGQSPKLLIYSASSRYTGVPSRFTGSGSGPDFTFTISSVQAEDLAVYFCQQHFRTPFTFGSGTKLEIK

SEQ ID NO: 14 - DNA, 726 bp, Artificial Sequence
atgcaggtacaactgcagcagtcaggacctgaactgaagaagcctggagagacagtcaagatctcctgcaaggcctctgggtatcctttcacaaactatggaatgaactgggtgaagcaggctccaggacagggtttaaagtggatgggctggattaacacctccactggagagtcaacatttgctgatgacttcaagggacggtttgacttctctttggaaacctctgccaacactgcctatttgcagatcaacaacctcaaaagtgaagactcggctacatatttctgtgcaagatgggaggtttaccacggctacgttccttactggggccaagggaccacggtcaccgtttcctctggcggtggcggttctggtggcggtggctccggcggtggcggttctgacatccagctgacccagtctcacaaattcctgtccacttcagtaggagacagggtcagcatcacctgcaaggccagtcaggatgtgtataatgctgttgcctggtatcaacagaaaccaggacaatctcctaaacttctgatttactcggcatcctcccggtacactggagtcccttctcgcttcactggcagtggctctgggccggatttcactttcaccatcagcagtgtgcaggctgaagacctggcagtttatttctgtcagcaacattttcgtactccattcacgttcggctcggggacaaaattggagatcaaa

SEQ ID NO: 15 - protein, 108 aa, Artificial Sequence
KIEVMYPPPYLDNEKSNGTIIHVKGKHLCPSPLFPGPSKPFWVLVVVGGVLACYSLLVTVAFIIFWVRSKRSRLLHSDYMNMTPRRPGPTRKHYQPYAPPRDFAAYRS

SEQ ID NO: 16 - DNA, 324 bp, Artificial Sequence
aaaattgaagttatgtatcctcctccttacctagacaatgagaagagcaatggaaccattatccatgtgaaagggaaacacctttgtccaagtcccctatttcccggaccttctaagcccttttgggtgctggtggtggttggtggagtcctggcttgctatagcttgctagtaacagtggcctttattattttctgggtgaggagtaagaggagcaggctcctgcacagtgactacatgaacatgactccccgccgccccgggcccacccgcaagcattaccagccctatgccccaccacgcgacttcgcagcctatcgctcc

SEQ ID NO: 17 - protein, 104 aa, Artificial Sequence
APAYQQGQNQLYNELNLGRREEYDVLDKRRGRDPEMGGKPQRRKNPQEGLYNELQKDKMAEAYSEIGMKGERRRGKGHDGLYQGLSTATKDTYDALHMQALPPR

SEQ ID NO: 18 - DNA, 315 bp, Artificial Sequence
gcccccgcgtaccagcagggccagaaccagctctataacgagctcaatctaggacgaagagaggagtacgatgttttggacaagagacgtggccgggaccctgagatggggggaaagccgcagagaaggaagaaccctcaggaaggcctgtacaatgaactgcagaaagataagatggcggaggcctacagtgagattgggatgaaaggcgagcgccggaggggcaaggggcacgatggcctttaccagggtctcagtacagccaccaaggacacctacgacgcccttcacatgcaggccctgccccctcgctaa

SEQ ID NO: 19 - protein, 26 aa, Artificial Sequence
RRKRSGSGEGRGSLLTCGDVEENPGP

SEQ ID NO: 20 - DNA, 78 bp, Artificial Sequence
agcggcagcggcgagggaagaggaagcctgctgacctgcggcgatgtggaggagaatcccggccccaggaggaagaga

SEQ ID NO: 21 - protein, 240 aa, Artificial Sequence
DIQMTQSPSSLSASVGDRVTITCRASQDVSTAVAWYQQKPGKAPKLLIYSASFLYSGVPSRFSGSGSGTDFTLTISSLQPEDFATYYCQQYLYHPATFGQGTKVEIKGGGGSGGGGSGGGGSEVQLVESGGGLVQPGGSLRLSCAASGFTFSDSWIHWVRQAPGKGLEWVAWISPYGGSTYYADSVKGRFTISADTSKNTAYLQMNSLRAEDTAVYYCARRHWPGGFDYWGQGTLVTVSA

SEQ ID NO: 22 - DNA, 720 bp, Artificial Sequence
gacatccaaatgacccagagccctagctccctgtccgctagcgtgggcgacagggtgaccatcacctgcagagccagccaggacgtgagcaccgccgtggcctggtaccagcagaagcccggcaaggcccccaagctgctgatctacagcgcctccttcctgtactccggcgtgccctccagatttagcggcagcggcagcggcacagacttcaccctcaccatcagctccctgcagcctgaggacttcgccacatactactgccagcagtacctctaccaccctgccaccttcggccaaggcaccaaggtggagatcaagggcggcggaggttctggcggaggcggctccggaggaggaggcagcgaagtgcagctggtggagagcggaggaggactggtgcagcctggcggaagcctgaggctgagctgtgctgccagcggcttcaccttctccgactcctggattcattgggtcaggcaggcccccggaaaaggactggagtgggtcgcctggatctccccttacggcggcagcacctactacgccgacagcgtgaagggcaggttcaccatcagcgccgataccagcaagaacaccgcctacctgcagatgaactccctgagggctgaggacaccgccgtgtactactgcgccaggaggcactggcctggcggattcgactactggggccagggcaccctggtgaccgtgtccgcc

SEQ ID NO: 23 - protein, 91 aa, Artificial Sequence
AAAFVPVFLPAKPTTTPAPRPPTPAPTIASQPLSLRPEACRPAAGGAVHTRGLDFACDIYIWAPLAGTCGVLLLSLVITLYCNHRNRFSVV

SEQ ID NO: 24 - DNA, 273 bp, Artificial Sequence
gcggccgcattcgtgccggtcttcctgccagcgaagcccaccacgacgccagcgccgcgaccaccaacaccggcgcccaccatcgcgtcgcagcccctgtccctgcgcccagaggcgtgccggccagcggcggggggcgcagtgcacacgagggggctggacttcgcctgtgatatctacatctgggcgcccttggccgggacttgtggggtccttctcctgtcactggttatcaccctttactgcaaccacaggaaccgtttctctgttgtt

SEQ ID NO: 25 - protein, 42 aa, Artificial Sequence
KRGRKKLLYIFKQPFMRPVQTTQEEDGCSCRFPEEEEGGCEL

SEQ ID NO: 26 - DNA, 126 bp, Artificial Sequence
aaacggggcagaaagaaactcctgtatatattcaaacaaccatttatgagaccagtacaaactactcaagaggaagatggctgtagctgccgatttccagaagaagaagaaggaggatgtgaactg